European Patent Application EP 4 682 158 A1, published January 21, 2026. Title: Cyclic peptide or salt thereof and use thereof. Applicant: FUJIFILM Corporation. Application WO. The sequence listing filed with the application follows.

SEQUENCE LISTING (463 sequences)

SEQ ID NO: 1 - DNA, 196 bp, synthetic construct
  misc_feature 1..196: note = Description of Artificial Sequence: Artificial DNA
  source 1..196: mol_type = other DNA
gaaattaatacgactcactatagggagaccacaacggtttccctctagaaataattttgtttaactttaagaaggagatatacatatggttaagaaaacaaaaacannntgtnnnnnnnnnnnnnnnnnntagnnnggtggctctggcggtagcaggacggggggcggcggggggtaaataaataagcttgagtat

SEQ ID NO: 2 - DNA, 105 bp, synthetic construct
  misc_feature 1..105: note = Description of Artificial Sequence: Artificial DNA
  source 1..105: mol_type = other DNA
gaaattaatacgactcactatagggagaccacaacggtttccctctagaaataattttgtttaactttaagaaggagatatacatatggttaaaaaaacaaaaac

SEQ ID NO: 3 - DNA, 63 bp, synthetic construct
  misc_feature 1..63: note = Description of Artificial Sequence: Artificial DNA
  source 1..63: mol_type = other DNA
atactcaagcttatttatttattaccccccgccgccccccgtcctgctaccgccagaaccacc

SEQ ID NO: 4 - DNA, 86 bp, synthetic construct
  misc_feature 1..86: note = Description of Artificial Sequence: Artificial DNA
  source 1..86: mol_type = other DNA
aagaaggagatatacatatggttaaaaaaacaaaaacannntgtnnnnnnnnnnnnnnnnnntagnnnggcggttctggcggtagc

SEQ ID NO: 5 - DNA, 89 bp, synthetic construct
  misc_feature 1..89: note = Description of Artificial Sequence: Artificial DNA
  source 1..89: mol_type = other DNA
aagaaggagatatacatatggttaaaaaaacaaaaacannntgtnnnnnnnnnnnnnnnnnnnnntagnnnggcggttctggcggtagc

SEQ ID NO: 6 - DNA, 92 bp, synthetic construct
  misc_feature 1..92: note = Description of Artificial Sequence: Artificial DNA
  source 1..92: mol_type = other DNA
aagaaggagatatacatatggttaaaaaaacaaaaacannntgtnnnnnnnnnnnnnnnnnnnnnnnntagnnnggcggttctggcggtagc

SEQ ID NO: 7 - DNA, 95 bp, synthetic construct
  misc_feature 1..95: note = Description of Artificial Sequence: Artificial DNA
  source 1..95: mol_type = other DNA
aagaaggagatatacatatggttaaaaaaacaaaaacannntgtnnnnnnnnnnnnnnnnnnnnnnnnnnntagnnnggcggttctggcggtagc

SEQ ID NO: 8 - DNA, 98 bp, synthetic construct
  misc_feature 1..98: note = Description of Artificial Sequence: Artificial DNA
  source 1..98: mol_type = other DNA
aagaaggagatatacatatggttaaaaaaacaaaaacannntgtnnnnnnnnnnnnnnnnnnnnnnnnnnnnnntagnnnggcggttctggcggtagc

SEQ ID NO: 9 - DNA, 101 bp, synthetic construct
  misc_feature 1..101: note = Description of Artificial Sequence: Artificial DNA
  source 1..101: mol_type = other DNA
aagaaggagatatacatatggttaaaaaaacaaaaacannntgtnnnnnnnnnnnnnnnnnnnnnnnnnnnnnnnnntagnnnggcggttctggcggtagc

SEQ ID NO: 10 - DNA, 104 bp, synthetic construct
  misc_feature 1..104: note = Description of Artificial Sequence: Artificial DNA
  source 1..104: mol_type = other DNA
aagaaggagatatacatatggttaaaaaaacaaaaacannntgtnnnnnnnnnnnnnnnnnnnnnnnnnnnnnnnnnnnntagnnnggcggttctggcggtagc

SEQ ID NO: 11 - DNA, 107 bp, synthetic construct
  misc_feature 1..107: note = Description of Artificial Sequence: Artificial DNA
  source 1..107: mol_type = other DNA
aagaaggagatatacatatggttaaaaaaacaaaaacannntgtnnnnnnnnnnnnnnnnnnnnnnnnnnnnnnnnnnnnnnntagnnnggcggttctggcggtagc

SEQ ID NO: 12 - DNA, 110 bp, synthetic construct
  misc_feature 1..110: note = Description of Artificial Sequence: Artificial DNA
  source 1..110: mol_type = other DNA
aagaaggagatatacatatggttaaaaaaacaaaaacannntgtnnnnnnnnnnnnnnnnnnnnnnnnnnnnnnnnnnnnnnnnnntagnnnggcggttctggcggtagc

SEQ ID NO: 13 - DNA, 113 bp, synthetic construct
  misc_feature 1..113: note = Description of Artificial Sequence: Artificial DNA
  source 1..113: mol_type = other DNA
aagaaggagatatacatatggttaaaaaaacaaaaacannntgtnnnnnnnnnnnnnnnnnnnnnnnnnnnnnnnnnnnnnnnnnnnnntagnnnggcggttctggcggtagc

SEQ ID NO: 14 - DNA, 116 bp, synthetic construct
  misc_feature 1..116: note = Description of Artificial Sequence: Artificial DNA
  source 1..116: mol_type = other DNA
aagaaggagatatacatatggttaaaaaaacaaaaacannntgtnnnnnnnnnnnnnnnnnnnnnnnnnnnnnnnnnnnnnnnnnnnnnnnntagnnnggcggttctggcggtagc

SEQ ID NO: 15 - DNA, 119 bp, synthetic construct
  misc_feature 1..119: note = Description of Artificial Sequence: Artificial DNA
  source 1..119: mol_type = other DNA
aagaaggagatatacatatggttaaaaaaacaaaaacannntgtnnnnnnnnnnnnnnnnnnnnnnnnnnnnnnnnnnnnnnnnnnnnnnnnnnntagnnnggcggttctggcggtagc

SEQ ID NO: 16 - DNA, 122 bp, synthetic construct
  misc_feature 1..122: note = Description of Artificial Sequence: Artificial DNA
  source 1..122: mol_type = other DNA
aagaaggagatatacatatggttaaaaaaacaaaaacannntgtnnnnnnnnnnnnnnnnnnnnnnnnnnnnnnnnnnnnnnnnnnnnnnnnnnnnnntagnnnggcggttctggcggtagc

SEQ ID NO: 17 - RNA, 23 nt, synthetic construct
  misc_feature 1..23: note = Description of Artificial Sequence: Artificial RNA
  source 1..23: mol_type = other RNA
taccccccgccgccccccgtcct

SEQ ID NO: 18 - DNA, 123 bp, synthetic construct
  misc_feature 1..123: note = Description of Artificial Sequence: Artificial DNA
  source 1..123: mol_type = other DNA
gttgtaaaacgacggccagtgccaagcttgggctaatacgactcactatagggagagtagttcaatggtagaacgtcggtctctaaaaccgagcgttgagggttcgattcctttctctcccac

SEQ ID NO: 19 - DNA, 18 bp, synthetic construct
  misc_feature 1..18: note = Description of Artificial Sequence: Artificial DNA
  source 1..18: mol_type = other DNA
gctaccgccagaaccacc

SEQ ID NO: 20 - DNA, 32 bp, synthetic construct
  misc_feature 1..32: note = Description of Artificial Sequence: Artificial DNA
  source 1..32: mol_type = other DNA
ggagatatacatatggttaagaaaacaaaaac

SEQ ID NO: 21 - DNA, 20 bp, synthetic construct
  misc_feature 1..20: note = Description of Artificial Sequence: Artificial DNA
  source 1..20: mol_type = other DNA
ctgctaccgccagaaccacc

SEQ ID NO: 22 - protein, 6 aa, synthetic construct
  REGION 1..6: note = Description of Artificial Sequence: Artificial peptide
VKKTKT

SEQ ID NO: 23 - protein, 10 aa, synthetic construct
  REGION 1..10: note = Description of Artificial Sequence: Artificial peptide
EQKLISEEDL

SEQ ID NO: 24 - protein, 11 aa, synthetic construct
  REGION 1..11: note = Description of Artificial Sequence: Artificial peptide
VSGWRLFKKIS

SEQ ID NO: 25 - protein, 57 aa, synthetic construct
  REGION 1..57: note = Description of Artificial Sequence: Artificial peptide
MVKKTKTHCSYERLQFHGHEAPFRVXVGSGSGSEQKLISEEDLGGSVSGWRLFKKIS

SEQ ID NO: 26 - DNA, 273 bp, synthetic construct
  misc_feature 1..273: note = Description of Artificial Sequence: Artificial DNA
  source 1..273: mol_type = other DNA
gaaattaatacgactcactatagggagaccacaacggtttccctctagaaataattttgtttaactttaagaaggagatataccaatggttaaaaaaacaaaaacacattgctcttacgaacgtctgcagttccatggtcatgaagctccgttccgtgtttaggttggttctggcagtggttccgaacagaaactgatcagcgaagaagatctgggtggctctgtaagtggatggcgattattcaagaagattagctaatgaataactaatcc

SEQ ID NO: 27 - DNA, 24 bp, synthetic construct
  misc_feature 1..24: note = Description of Artificial Sequence: Artificial DNA
  source 1..24: mol_type = other DNA
gaaattaatacgactcactatagg

SEQ ID NO: 28 - DNA, 17 bp, synthetic construct
  misc_feature 1..17: note = Description of Artificial Sequence: Artificial DNA
  source 1..17: mol_type = other DNA
gaaccactgccagaacc

SEQ ID NO: 29 - DNA, 105 bp, synthetic construct
  misc_feature 1..105: note = Description of Artificial Sequence: Artificial DNA
  source 1..105: mol_type = other DNA
gaaattaatacgactcactatagggagaccacaacggtttccctctagaaataattttgtttaactttaagaaggagatataccaatggttaaaaaaacaaaaac

SEQ ID NO: 30 - DNA, 95 bp, synthetic construct
  misc_feature 1..95: note = Description of Artificial Sequence: Artificial DNA
  source 1..95: mol_type = other DNA
gaaccactgccagaaccaacctaaacacggaacggagcttcatgaccatggaactgcagacgttcgtaagagcaatgtgtttttgtttttttaac

SEQ ID NO: 31 - DNA, 24 bp, synthetic construct
  misc_feature 1..24: note = Description of Artificial Sequence: Artificial DNA
  source 1..24: mol_type = other DNA
ggattagttattcattagctaatc

SEQ ID NO: 32 - DNA, 107 bp, synthetic construct
  misc_feature 1..107: note = Description of Artificial Sequence: Artificial DNA
  source 1..107: mol_type = other DNA
ggttctggcagtggttccgaacagaaactgatcagcgaagaagatctgggtggctctgtaagtggatggcgattattcaagaagattagctaatgaataactaatcc

SEQ ID NO: 33 - protein, 24 aa, synthetic construct
  REGION 1..24: note = Description of Artificial Sequence: Artificial peptide
EQKLISEEDLGGSVSGWRLFKKIS

SEQ ID NO: 34 - protein, 15 aa, synthetic construct
  REGION 1..15: note = Description of Artificial Sequence: Cyclic peptide
CRALLRGAPFHLAEC

SEQ ID NO: 35 - protein, 15 aa, synthetic construct
  REGION 1..15: note = Description of Artificial Sequence: Cyclic peptide
YRSRKYSSWYVALKR

SEQ ID NO: 36 - protein, 15 aa, synthetic construct
  REGION 1..15: note = Description of Artificial Sequence: Cyclic peptide
CRALLRGAPFHLAEK

SEQ ID NO: 37 - protein, 20 aa, synthetic construct
  REGION 1..20: note = Description of Artificial Sequence: Cyclic peptide
QCQLNYWDDLQFTYYLQYKV

SEQ ID NO: 38 - protein, 20 aa, synthetic construct
  REGION 1..20: note = Description of Artificial Sequence: Cyclic peptide
QCSYLYQYVFERYKVTVPKD

SEQ ID NO: 39 - protein, 19 aa, synthetic construct
  REGION 1..19: note = Description of Artificial Sequence: Cyclic peptide
QCENWLSQDQWKYFWQYKI

SEQ ID NO: 40 - protein, 20 aa, synthetic construct
  REGION 1..20: note = Description of Artificial Sequence: Cyclic peptide
DCSGNFFSKEQFHYLELFKK

SEQ ID NO: 41 - protein, 19 aa, synthetic construct
  REGION 1..19: note = Description of Artificial Sequence: Cyclic peptide
LCGNYITPLQWKYFQTYKW

SEQ ID NO: 42 - protein, 18 aa, synthetic construct
  REGION 1..18: note = Description of Artificial Sequence: Cyclic peptide
QCYFLSQYILERYKVHKL

SEQ ID NO: 43 - protein, 20 aa, synthetic construct
  REGION 1..20: note = Description of Artificial Sequence: Cyclic peptide
HCNANFVYQQQYLYLLQYKL

SEQ ID NO: 44 - protein, 20 aa, synthetic construct
  REGION 1..20: note = Description of Artificial Sequence: Cyclic peptide
ACEYNYWNQVQFTFLIAFKR

SEQ ID NO: 45 - protein, 20 aa, synthetic construct
  REGION 1..20: note = Description of Artificial Sequence: Cyclic peptide
TCPQNFRDELQFTYFTQYKY

SEQ ID NO: 46 - protein, 20 aa, synthetic construct
  REGION 1..20: note = Description of Artificial Sequence: Cyclic peptide
SCIQQNYFWQYVFERYRYKQ

SEQ ID NO: 47 - protein, 20 aa, synthetic construct
  REGION 1..20: note = Description of Artificial Sequence: Cyclic peptide
KCPQNFINPVQWRYFQHYKN

SEQ ID NO: 48 - protein, 17 aa, synthetic construct
  REGION 1..17: note = Description of Artificial Sequence: Cyclic peptide
GCYWNEVQYYYLQQYKQ

SEQ ID NO: 49 - protein, 20 aa, synthetic construct
  REGION 1..20: note = Description of Artificial Sequence: Cyclic peptide
SCQGNWISNTQFRYFIAYKT

SEQ ID NO: 50 - protein, 20 aa, synthetic construct
  REGION 1..20: note = Description of Artificial Sequence: Cyclic peptide
ACGQNFYHPVQFHYFIAYKQ

SEQ ID NO: 51 - protein, 20 aa, synthetic construct
  REGION 1..20: note = Description of Artificial Sequence: Cyclic peptide
VCHSNFLSAVQYAYFYQYKH

SEQ ID NO: 52 - protein, 20 aa, synthetic construct
  REGION 1..20: note = Description of Artificial Sequence: Cyclic peptide
VCNENNWSRSQYHFFLQYKY

SEQ ID NO: 53 - protein, 20 aa, synthetic construct
  REGION 1..20: note = Description of Artificial Sequence: Cyclic peptide
ACPQNFINPVQWRYFQHYKN

SEQ ID NO: 54 - protein, 20 aa, synthetic construct
  REGION 1..20: note = Description of Artificial Sequence: Cyclic peptide
KCAQNFINPVQWRYFQHYKN

SEQ ID NO: 55 - protein, 20 aa, synthetic construct
  REGION 1..20: note = Description of Artificial Sequence: Cyclic peptide
KCPANFINPVQWRYFQHYKN

SEQ ID NO: 56 - protein, 20 aa, synthetic construct
  REGION 1..20: note = Description of Artificial Sequence: Cyclic peptide
KCPQAFINPVQWRYFQHYKN

SEQ ID NO: 57 - protein, 20 aa, synthetic construct
  REGION 1..20: note = Description of Artificial Sequence: Cyclic peptide
KCPQNAINPVQWRYFQHYKN

SEQ ID NO: 58 - protein, 20 aa, synthetic construct
  REGION 1..20: note = Description of Artificial Sequence: Cyclic peptide
KCPQNFANPVQWRYFQHYKN

SEQ ID NO: 59 - protein, 20 aa, synthetic construct
  REGION 1..20: note = Description of Artificial Sequence: Cyclic peptide
KCPQNFIAPVQWRYFQHYKN

SEQ ID NO: 60 - protein, 20 aa, synthetic construct
  REGION 1..20: note = Description of Artificial Sequence: Cyclic peptide
KCPQNFINAVQWRYFQHYKN

SEQ ID NO: 61 - protein, 20 aa, synthetic construct
  REGION 1..20: note = Description of Artificial Sequence: Cyclic peptide
KCPQNFINPAQWRYFQHYKN

SEQ ID NO: 62 - protein, 20 aa, synthetic construct
  REGION 1..20: note = Description of Artificial Sequence: Cyclic peptide
KCPQNFINPVQARYFQHYKN

SEQ ID NO: 63 - protein, 20 aa, synthetic construct
  REGION 1..20: note = Description of Artificial Sequence: Cyclic peptide
KCPQNFINPVQWAYFQHYKN

SEQ ID NO: 64 - protein, 20 aa, synthetic construct
  REGION 1..20: note = Description of Artificial Sequence: Cyclic peptide
KCPQNFINPVQWRAFQHYKN

SEQ ID NO: 65 - protein, 20 aa, synthetic construct
  REGION 1..20: note = Description of Artificial Sequence: Cyclic peptide
KCPQNFINPVQWRYFAHYKN

SEQ ID NO: 66 - protein, 20 aa, synthetic construct
  REGION 1..20: note = Description of Artificial Sequence: Cyclic peptide
KCPQNFINPVQWRYFQAYKN

SEQ ID NO: 67 - protein, 20 aa, synthetic construct
  REGION 1..20: note = Description of Artificial Sequence: Cyclic peptide
KCPQNFINPVQWRYFQHYKA

SEQ ID NO: 68 - protein, 19 aa, synthetic construct
  REGION 1..19: note = Description of Artificial Sequence: Cyclic peptide
KCQNFINPVQWRYFQHYKN

SEQ ID NO: 69 - protein, 21 aa, synthetic construct
  REGION 1..21: note = Description of Artificial Sequence: Cyclic peptide
KCPQNFINPVQWRYFQHYAKN

SEQ ID NO: 70 - protein, 21 aa, synthetic construct
  REGION 1..21: note = Description of Artificial Sequence: Cyclic peptide
KCAPQNFINPVQWRYFQHYKN

SEQ ID NO: 71 - protein, 20 aa, synthetic construct
  REGION 1..20: note = Description of Artificial Sequence: Cyclic peptide
GCPQNFINPVQWRYFQHYKN

SEQ ID NO: 72 - protein, 20 aa, synthetic construct
  REGION 1..20: note = Description of Artificial Sequence: Cyclic peptide
PCPQNFINPVQWRYFQHYKN

SEQ ID NO: 73 - protein, 20 aa, synthetic construct
  REGION 1..20: note = Description of Artificial Sequence: Cyclic peptide
LCPQNFINPVQWRYFQHYKN

SEQ ID NO: 74 - protein, 20 aa, synthetic construct
  REGION 1..20: note = Description of Artificial Sequence: Cyclic peptide
ICPQNFINPVQWRYFQHYKN

SEQ ID NO: 75 - protein, 20 aa, synthetic construct
  REGION 1..20: note = Description of Artificial Sequence: Cyclic peptide
VCPQNFINPVQWRYFQHYKN

SEQ ID NO: 76 - protein, 20 aa, synthetic construct
  REGION 1..20: note = Description of Artificial Sequence: Cyclic peptide
FCPQNFINPVQWRYFQHYKN

SEQ ID NO: 77 - protein, 20 aa, synthetic construct
  REGION 1..20: note = Description of Artificial Sequence: Cyclic peptide
YCPQNFINPVQWRYFQHYKN

SEQ ID NO: 78 - protein, 20 aa, synthetic construct
  REGION 1..20: note = Description of Artificial Sequence: Cyclic peptide
WCPQNFINPVQWRYFQHYKN

SEQ ID NO: 79 - protein, 20 aa, synthetic construct
  REGION 1..20: note = Description of Artificial Sequence: Cyclic peptide
NCPQNFINPVQWRYFQHYKN

SEQ ID NO: 80 - protein, 20 aa, synthetic construct
  REGION 1..20: note = Description of Artificial Sequence: Cyclic peptide
QCPQNFINPVQWRYFQHYKN

SEQ ID NO: 81 - protein, 20 aa, synthetic construct
  REGION 1..20: note = Description of Artificial Sequence: Cyclic peptide
SCPQNFINPVQWRYFQHYKN

SEQ ID NO: 82 - protein, 20 aa, synthetic construct
  REGION 1..20: note = Description of Artificial Sequence: Cyclic peptide
TCPQNFINPVQWRYFQHYKN

SEQ ID NO: 83 - protein, 20 aa, synthetic construct
  REGION 1..20: note = Description of Artificial Sequence: Cyclic peptide
DCPQNFINPVQWRYFQHYKN

SEQ ID NO: 84 - protein, 20 aa, synthetic construct
  REGION 1..20: note = Description of Artificial Sequence: Cyclic peptide
ECPQNFINPVQWRYFQHYKN

SEQ ID NO: 85 - protein, 20 aa, synthetic construct
  REGION 1..20: note = Description of Artificial Sequence: Cyclic peptide
RCPQNFINPVQWRYFQHYKN

SEQ ID NO: 86 - protein, 20 aa, synthetic construct
  REGION 1..20: note = Description of Artificial Sequence: Cyclic peptide
HCPQNFINPVQWRYFQHYKN

SEQ ID NO: 87 - protein, 20 aa, synthetic construct
  REGION 1..20: note = Description of Artificial Sequence: Cyclic peptide
QCPQNFINPVHWRYFQHYKN

SEQ ID NO: 88 - protein, 20 aa, synthetic construct
  REGION 1..20: note = Description of Artificial Sequence: Cyclic peptide
QCPQNFINPVQWRYLQHYKN

SEQ ID NO: 89 - protein, 20 aa, synthetic construct
  REGION 1..20: note = Description of Artificial Sequence: Cyclic peptide
QCPQNFINPVQWRYYQHYKN

SEQ ID NO: 90 - protein, 20 aa, synthetic construct
  REGION 1..20: note = Description of Artificial Sequence: Cyclic peptide
QCPQNFINPVQWRYRQHYKN

SEQ ID NO: 91 - protein, 20 aa, synthetic construct
  REGION 1..20: note = Description of Artificial Sequence: Cyclic peptide
QCPQNFINPVQWRYFQHVKN

SEQ ID NO: 92 - protein, 20 aa, synthetic construct
  REGION 1..20: note = Description of Artificial Sequence: Cyclic peptide
QCPQNFINPVQWRYFQHFKN

SEQ ID NO: 93 - protein, 20 aa, synthetic construct
  REGION 1..20: note = Description of Artificial Sequence: Cyclic peptide
QCPQNFINPVQWRYFQHWKN

SEQ ID NO: 94 - protein, 20 aa, synthetic construct
  REGION 1..20: note = Description of Artificial Sequence: Cyclic peptide
QCPQNFINPVQWRYFQHSKN

SEQ ID NO: 95 - protein, 20 aa, synthetic construct
  REGION 1..20: note = Description of Artificial Sequence: Cyclic peptide
QCPQGFINPVQWRYFQHYKN

SEQ ID NO: 96 - protein, 20 aa, synthetic construct
  REGION 1..20: note = Description of Artificial Sequence: Cyclic peptide
QCPQYFINPVQWRYFQHYKN

SEQ ID NO: 97 - protein, 20 aa, synthetic construct
  REGION 1..20: note = Description of Artificial Sequence: Cyclic peptide
QCPQSFINPVQWRYFQHYKN

SEQ ID NO: 98 - protein, 20 aa, synthetic construct
  REGION 1..20: note = Description of Artificial Sequence: Cyclic peptide
QCPQTFINPVQWRYFQHYKN

SEQ ID NO: 99 - protein, 20 aa, synthetic construct
  REGION 1..20: note = Description of Artificial Sequence: Cyclic peptide
QCPQEFINPVQWRYFQHYKN

SEQ ID NO: 100 - protein, 20 aa, synthetic construct
  REGION 1..20: note = Description of Artificial Sequence: Cyclic peptide
QCPQHFINPVQWRYFQHYKN

SEQ ID NO: 101 - protein, 20 aa, synthetic construct
  REGION 1..20: note = Description of Artificial Sequence: Cyclic peptide
QCPQNFINPVQIRYFQHYKN

SEQ ID NO: 102 - protein, 20 aa, synthetic construct
  REGION 1..20: note = Description of Artificial Sequence: Cyclic peptide
QCPQNFINPVQVRYFQHYKN

SEQ ID NO: 103 - protein, 20 aa, synthetic construct
  REGION 1..20: note = Description of Artificial Sequence: Cyclic peptide
QCPQNFINPVQFRYFQHYKN

SEQ ID NO: 104 - protein, 20 aa, synthetic construct
  REGION 1..20: note = Description of Artificial Sequence: Cyclic peptide
QCPQNFINPVQYRYFQHYKN

SEQ ID NO: 105 - protein, 20 aa, synthetic construct
  REGION 1..20: note = Description of Artificial Sequence: Cyclic peptide
QCPQNFINPVQSRYFQHYKN

SEQ ID NO: 106 - protein, 20 aa, synthetic construct
  REGION 1..20: note = Description of Artificial Sequence: Cyclic peptide
QCPQNFINPVQHRYFQHYKN

SEQ ID NO: 107 - protein, 20 aa, synthetic construct
  REGION 1..20: note = Description of Artificial Sequence: Cyclic peptide
YCTDNYIDDIQFWYLFLYKQ

SEQ ID NO: 108 - protein, 19 aa, synthetic construct
  REGION 1..19: note = Description of Artificial Sequence: Cyclic peptide
LCRNYINPQQWRYFALYKY

SEQ ID NO: 109 - protein, 17 aa, synthetic construct
  REGION 1..17: note = Description of Artificial Sequence: Cyclic peptide
DCFINELQYFYIQQYKK

SEQ ID NO: 110 - protein, 20 aa, synthetic construct
  REGION 1..20: note = Description of Artificial Sequence: Cyclic peptide
QCQTDHQQQLYFIYQYLQKI

SEQ ID NO: 111 - protein, 20 aa, synthetic construct
  REGION 1..20: note = Description of Artificial Sequence: Cyclic peptide
QCDQEFYLALYAWTLRSYKL

SEQ ID NO: 112 - protein, 20 aa, synthetic construct
  REGION 1..20: note = Description of Artificial Sequence: Cyclic peptide
HCQPEYELYYIYLYLNALKI

SEQ ID NO: 113 - protein, 19 aa, synthetic construct
  REGION 1..19: note = Description of Artificial Sequence: Cyclic peptide
RCINYWSGQQFYFFQQYKF

SEQ ID NO: 114 - protein, 20 aa, synthetic construct
  REGION 1..20: note = Description of Artificial Sequence: Cyclic peptide
YCTDNYIDDIQFWYLFLYKH

SEQ ID NO: 115 - protein, 19 aa, synthetic construct
  REGION 1..19: note = Description of Artificial Sequence: Cyclic peptide
NCPNYWSQIQWHYFQAYKQ

SEQ ID NO: 116 - protein, 19 aa, synthetic construct
  REGION 1..19: note = Description of Artificial Sequence: Cyclic peptide
QCYQNWYLYQYLVERYYKD

SEQ ID NO: 117 - protein, 19 aa, synthetic construct
  REGION 1..19: note = Description of Artificial Sequence: Cyclic peptide
LCRNYINPQQWRYFALYKN

SEQ ID NO: 118 - protein, 20 aa, synthetic construct
  REGION 1..20: note = Description of Artificial Sequence: Cyclic peptide
LCPVPQQTDYLRWYQIIHKQ

SEQ ID NO: 119 - protein, 20 aa, synthetic construct
  REGION 1..20: note = Description of Artificial Sequence: Cyclic peptide
QCRYFWQYVLERYRVRLPKE

SEQ ID NO: 120 - protein, 20 aa, synthetic construct
  REGION 1..20: note = Description of Artificial Sequence: Cyclic peptide
QCWYIQQYIWERYFLWHNKE

SEQ ID NO: 121 - protein, 17 aa, synthetic construct
  REGION 1..17: note = Description of Artificial Sequence: Cyclic peptide
DCYWDDQQYSFLQLYKR

SEQ ID NO: 122 - protein, 19 aa, synthetic construct
  REGION 1..19: note = Description of Artificial Sequence: Cyclic peptide
QCENWVNSTQFEFFWQYKT

SEQ ID NO: 123 - protein, 19 aa, synthetic construct
  REGION 1..19: note = Description of Artificial Sequence: Cyclic peptide
QCQNFITEVQFTYFWHYKT

SEQ ID NO: 124 - protein, 19 aa, synthetic construct
  REGION 1..19: note = Description of Artificial Sequence: Cyclic peptide
DCRDLQLFYIYQYLDALKK

SEQ ID NO: 125 - protein, 20 aa, synthetic construct
  REGION 1..20: note = Description of Artificial Sequence: Cyclic peptide
YCRDNYFYLEQWQYLYLYKH

SEQ ID NO: 126 - protein, 20 aa, synthetic construct
  REGION 1..20: note = Description of Artificial Sequence: Cyclic peptide
LCEINWLSQEQYGYFIEYKT

SEQ ID NO: 127 - protein, 20 aa, synthetic construct
  REGION 1..20: note = Description of Artificial Sequence: Cyclic peptide
YCPYNFYNIIQFHYFLTYKT

SEQ ID NO: 128 - protein, 20 aa, synthetic construct
  REGION 1..20: note = Description of Artificial Sequence: Cyclic peptide
PCVQNYFNDLQWIFLQHYKR

SEQ ID NO: 129 - protein, 20 aa, synthetic construct
  REGION 1..20: note = Description of Artificial Sequence: Cyclic peptide
ECPWNFVNQLQWQYFITYKV

SEQ ID NO: 130 - protein, 20 aa, synthetic construct
  REGION 1..20: note = Description of Artificial Sequence: Cyclic peptide
HCDGNWWNSQQFFYLLLYKH

SEQ ID NO: 131 - protein, 20 aa, synthetic construct
  REGION 1..20: note = Description of Artificial Sequence: Cyclic peptide
YCEENYLDPEQYQYFIYFKY

SEQ ID NO: 132 - protein, 20 aa, synthetic construct
  REGION 1..20: note = Description of Artificial Sequence: Cyclic peptide
ECQENFVDRQQYWYFLSYKF

SEQ ID NO: 133 - protein, 20 aa, synthetic construct
  REGION 1..20: note = Description of Artificial Sequence: Cyclic peptide
ECLGNYFSHEQYQYLLQYKI

SEQ ID NO: 134 - protein, 20 aa, synthetic construct
  REGION 1..20: note = Description of Artificial Sequence: Cyclic peptide
LCADQYDYLLQYVFWRTYKI

SEQ ID NO: 135 - protein, 18 aa, synthetic construct
  REGION 1..18: note = Description of Artificial Sequence: Cyclic peptide
QCTYLAQYLVERYHLTKT

SEQ ID NO: 136 - protein, 20 aa, synthetic construct
  REGION 1..20: note = Description of Artificial Sequence: Cyclic peptide
GCEENYLDPEQYQYFIYFKY

SEQ ID NO: 137 - protein, 20 aa, synthetic construct
  REGION 1..20: note = Description of Artificial Sequence: Cyclic peptide
PCEENYLDPEQYQYFIYFKY

SEQ ID NO: 138 - protein, 20 aa, synthetic construct
  REGION 1..20: note = Description of Artificial Sequence: Cyclic peptide
LCEENYLDPEQYQYFIYFKY

SEQ ID NO: 139 - protein, 20 aa, synthetic construct
  REGION 1..20: note = Description of Artificial Sequence: Cyclic peptide
ICEENYLDPEQYQYFIYFKY

SEQ ID NO: 140 - protein, 20 aa, synthetic construct
  REGION 1..20: note = Description of Artificial Sequence: Cyclic peptide
VCEENYLDPEQYQYFIYFKY

SEQ ID NO: 141 - protein, 20 aa, synthetic construct
  REGION 1..20: note = Description of Artificial Sequence: Cyclic peptide
FCEENYLDPEQYQYFIYFKY

SEQ ID NO: 142 - protein, 20 aa, synthetic construct
  REGION 1..20: note = Description of Artificial Sequence: Cyclic peptide
WCEENYLDPEQYQYFIYFKY

SEQ ID NO: 143 - protein, 20 aa, synthetic construct
  REGION 1..20: note = Description of Artificial Sequence: Cyclic peptide
NCEENYLDPEQYQYFIYFKY

SEQ ID NO: 144 - protein, 20 aa, synthetic construct
  REGION 1..20: note = Description of Artificial Sequence: Cyclic peptide
QCEENYLDPEQYQYFIYFKY

SEQ ID NO: 145 - protein, 20 aa, synthetic construct
  REGION 1..20: note = Description of Artificial Sequence: Cyclic peptide
SCEENYLDPEQYQYFIYFKY

SEQ ID NO: 146 - protein, 20 aa, synthetic construct
  REGION 1..20: note = Description of Artificial Sequence: Cyclic peptide
TCEENYLDPEQYQYFIYFKY

SEQ ID NO: 147 - protein, 20 aa, synthetic construct
  REGION 1..20: note = Description of Artificial Sequence: Cyclic peptide
DCEENYLDPEQYQYFIYFKY

SEQ ID NO: 148 - protein, 20 aa, synthetic construct
  REGION 1..20: note = Description of Artificial Sequence: Cyclic peptide
ECEENYLDPEQYQYFIYFKY

SEQ ID NO: 149 - protein, 20 aa, synthetic construct
  REGION 1..20: note = Description of Artificial Sequence: Cyclic peptide
RCEENYLDPEQYQYFIYFKY

SEQ ID NO: 150 - protein, 20 aa, synthetic construct
  REGION 1..20: note = Description of Artificial Sequence: Cyclic peptide
HCEENYLDPEQYQYFIYFKY

SEQ ID NO: 151 - protein, 20 aa, synthetic construct
  REGION 1..20: note = Description of Artificial Sequence: Cyclic peptide
YCGENYLDPEQYQYFIYFKY

SEQ ID NO: 152 - protein, 20 aa, synthetic construct
  REGION 1..20: note = Description of Artificial Sequence: Cyclic peptide
YCPENYLDPEQYQYFIYFKY

SEQ ID NO: 153 - protein, 20 aa, synthetic construct
  REGION 1..20: note = Description of Artificial Sequence: Cyclic peptide
YCLENYLDPEQYQYFIYFKY

SEQ ID NO: 154 - protein, 20 aa, synthetic construct
  REGION 1..20: note = Description of Artificial Sequence: Cyclic peptide
YCIENYLDPEQYQYFIYFKY

SEQ ID NO: 155 - protein, 20 aa, synthetic construct
  REGION 1..20: note = Description of Artificial Sequence: Cyclic peptide
YCVENYLDPEQYQYFIYFKY

SEQ ID NO: 156 - protein, 20 aa, synthetic construct
  REGION 1..20: note = Description of Artificial Sequence: Cyclic peptide
YCFENYLDPEQYQYFIYFKY

SEQ ID NO: 157 - protein, 20 aa, synthetic construct
  REGION 1..20: note = Description of Artificial Sequence: Cyclic peptide
YCYENYLDPEQYQYFIYFKY

SEQ ID NO: 158 - protein, 20 aa, synthetic construct
  REGION 1..20: note = Description of Artificial Sequence: Cyclic peptide
YCWENYLDPEQYQYFIYFKY

SEQ ID NO: 159 - protein, 20 aa, synthetic construct
  REGION 1..20: note = Description of Artificial Sequence: Cyclic peptide
YCNENYLDPEQYQYFIYFKY

SEQ ID NO: 160 - protein, 20 aa, synthetic construct
  REGION 1..20: note = Description of Artificial Sequence: Cyclic peptide
YCQENYLDPEQYQYFIYFKY

SEQ ID NO: 161 - protein, 20 aa, synthetic construct
  REGION 1..20: note = Description of Artificial Sequence: Cyclic peptide
YCSENYLDPEQYQYFIYFKY

SEQ ID NO: 162 - protein, 20 aa, synthetic construct
  REGION 1..20: note = Description of Artificial Sequence: Cyclic peptide
YCTENYLDPEQYQYFIYFKY

SEQ ID NO: 163 - protein, 20 aa, synthetic construct
  REGION 1..20: note = Description of Artificial Sequence: Cyclic peptide
YCDENYLDPEQYQYFIYFKY

SEQ ID NO: 164 - protein, 20 aa, synthetic construct
  REGION 1..20: note = Description of Artificial Sequence: Cyclic peptide
YCRENYLDPEQYQYFIYFKY

SEQ ID NO: 165 - protein, 20 aa, synthetic construct
  REGION 1..20: note = Description of Artificial Sequence: Cyclic peptide
YCHENYLDPEQYQYFIYFKY

SEQ ID NO: 166 - protein, 20 aa, synthetic construct
  REGION 1..20: note = Description of Artificial Sequence: Cyclic peptide
YCEGNYLDPEQYQYFIYFKY

SEQ ID NO: 167 - protein, 20 aa, synthetic construct
  REGION 1..20: note = Description of Artificial Sequence: Cyclic peptide
YCEPNYLDPEQYQYFIYFKY

SEQ ID NO: 168 - protein, 20 aa, synthetic construct
  REGION 1..20: note = Description of Artificial Sequence: Cyclic peptide
YCELNYLDPEQYQYFIYFKY

SEQ ID NO: 169 - protein, 20 aa, synthetic construct
  REGION 1..20: note = Description of Artificial Sequence: Cyclic peptide
YCEINYLDPEQYQYFIYFKY

SEQ ID NO: 170 - protein, 20 aa, synthetic construct
  REGION 1..20: note = Description of Artificial Sequence: Cyclic peptide
YCEVNYLDPEQYQYFIYFKY

SEQ ID NO: 171 - protein, 20 aa, synthetic construct
  REGION 1..20: note = Description of Artificial Sequence: Cyclic peptide
YCEFNYLDPEQYQYFIYFKY

SEQ ID NO: 172 - protein, 20 aa, synthetic construct
  REGION 1..20: note = Description of Artificial Sequence: Cyclic peptide
YCEYNYLDPEQYQYFIYFKY

SEQ ID NO: 173 - protein, 20 aa, synthetic construct
  REGION 1..20: note = Description of Artificial Sequence: Cyclic peptide
YCEWNYLDPEQYQYFIYFKY

SEQ ID NO: 174 - protein, 20 aa, synthetic construct
  REGION 1..20: note = Description of Artificial Sequence: Cyclic peptide
YCENNYLDPEQYQYFIYFKY

SEQ ID NO: 175 - protein, 20 aa, synthetic construct
  REGION 1..20: note = Description of Artificial Sequence: Cyclic peptide
YCEQNYLDPEQYQYFIYFKY

SEQ ID NO: 176 - protein, 20 aa, synthetic construct
  REGION 1..20: note = Description of Artificial Sequence: Cyclic peptide
YCESNYLDPEQYQYFIYFKY

SEQ ID NO: 177 - protein, 20 aa, synthetic construct
  REGION 1..20: note = Description of Artificial Sequence: Cyclic peptide
YCETNYLDPEQYQYFIYFKY

SEQ ID NO: 178 - protein, 20 aa, synthetic construct
  REGION 1..20: note = Description of Artificial Sequence: Cyclic peptide
YCEDNYLDPEQYQYFIYFKY

SEQ ID NO: 179 - protein, 20 aa, synthetic construct
  REGION 1..20: note = Description of Artificial Sequence: Cyclic peptide
YCERNYLDPEQYQYFIYFKY

SEQ ID NO: 180 - protein, 20 aa, synthetic construct
  REGION 1..20: note = Description of Artificial Sequence: Cyclic peptide
YCEHNYLDPEQYQYFIYFKY

SEQ ID NO: 181 - protein, 20 aa, synthetic construct
  REGION 1..20: note = Description of Artificial Sequence: Cyclic peptide
YCEEGYLDPEQYQYFIYFKY

SEQ ID NO: 182 - protein, 20 aa, synthetic construct
  REGION 1..20: note = Description of Artificial Sequence: Cyclic peptide
YCEEWYLDPEQYQYFIYFKY

SEQ ID NO: 183 - protein, 20 aa, synthetic construct
  REGION 1..20: note = Description of Artificial Sequence: Cyclic peptide
YCEEQYLDPEQYQYFIYFKY

SEQ ID NO: 184 - protein, 20 aa, synthetic construct
  REGION 1..20: note = Description of Artificial Sequence: Cyclic peptide
YCEESYLDPEQYQYFIYFKY

SEQ ID NO: 185 - protein, 20 aa, synthetic construct
  REGION 1..20: note = Description of Artificial Sequence: Cyclic peptide
YCEETYLDPEQYQYFIYFKY

SEQ ID NO: 186 - protein, 20 aa, synthetic construct
  REGION 1..20: note = Description of Artificial Sequence: Cyclic peptide
YCEENLLDPEQYQYFIYFKY

SEQ ID NO: 187 - protein, 20 aa, synthetic construct
  REGION 1..20: note = Description of Artificial Sequence: Cyclic peptide
YCEENFLDPEQYQYFIYFKY

SEQ ID NO: 188 - protein, 20 aa, synthetic construct
  REGION 1..20: note = Description of Artificial Sequence: Cyclic peptide
YCEENWLDPEQYQYFIYFKY

SEQ ID NO: 189 - protein, 20 aa, synthetic construct
  REGION 1..20: note = Description of Artificial Sequence: Cyclic peptide
YCEENNLDPEQYQYFIYFKY

SEQ ID NO: 190 - protein, 20 aa, synthetic construct
  REGION 1..20: note = Description of Artificial Sequence: Cyclic peptide
YCEENQLDPEQYQYFIYFKY

SEQ ID NO: 191 - protein, 20 aa, synthetic construct
  REGION 1..20: note = Description of Artificial Sequence: Cyclic peptide
YCEENSLDPEQYQYFIYFKY

SEQ ID NO: 192 - protein, 20 aa, synthetic construct
  REGION 1..20: note = Description of Artificial Sequence: Cyclic peptide
YCEENDLDPEQYQYFIYFKY

SEQ ID NO: 193 - protein, 20 aa, synthetic construct
  REGION 1..20: note = Description of Artificial Sequence: Cyclic peptide
YCEENRLDPEQYQYFIYFKY

SEQ ID NO: 194 - protein, 20 aa, synthetic construct
  REGION 1..20: note = Description of Artificial Sequence: Cyclic peptide
YCEENHLDPEQYQYFIYFKY

SEQ ID NO: 195 - protein, 20 aa, synthetic construct
  REGION 1..20: note = Description of Artificial Sequence: Cyclic peptide
YCEENYIDPEQYQYFIYFKY

SEQ ID NO: 196 - protein, 20 aa, synthetic construct
  REGION 1..20: note = Description of Artificial Sequence: Cyclic peptide
YCEENYVDPEQYQYFIYFKY

SEQ ID NO: 197 - protein, 20 aa, synthetic construct
  REGION 1..20: note = Description of Artificial Sequence: Cyclic peptide
YCEENYFDPEQYQYFIYFKY

SEQ ID NO: 198 - protein, 20 aa, synthetic construct
  REGION 1..20: note = Description of Artificial Sequence: Cyclic peptide
YCEENYYDPEQYQYFIYFKY

SEQ ID NO: 199 - protein, 20 aa, synthetic construct
  REGION 1..20: note = Description of Artificial Sequence: Cyclic peptide
YCEENYWDPEQYQYFIYFKY

SEQ ID NO: 200 - protein, 20 aa, synthetic construct
  REGION 1..20: note = Description of Artificial Sequence: Cyclic peptide
YCEENYNDPEQYQYFIYFKY

SEQ ID NO: 201 - protein, 20 aa, synthetic construct
  REGION 1..20: note = Description of Artificial Sequence: Cyclic peptide
YCEENYQDPEQYQYFIYFKY

SEQ ID NO: 202 - protein, 20 aa, synthetic construct
  REGION 1..20: note = Description of Artificial Sequence: Cyclic peptide
YCEENYSDPEQYQYFIYFKY

SEQ ID NO: 203 - protein, 20 aa, synthetic construct
  REGION 1..20: note = Description of Artificial Sequence: Cyclic peptide
YCEENYTDPEQYQYFIYFKY

SEQ ID NO: 204 - protein, 20 aa, synthetic construct
  REGION 1..20: note = Description of Artificial Sequence: Cyclic peptide
YCEENYEDPEQYQYFIYFKY

SEQ ID NO: 205 - protein, 20 aa, synthetic construct
  REGION 1..20: note = Description of Artificial Sequence: Cyclic peptide
YCEENYRDPEQYQYFIYFKY

SEQ ID NO: 206 - protein, 20 aa, synthetic construct
  REGION 1..20: note = Description of Artificial Sequence: Cyclic peptide
YCEENYHDPEQYQYFIYFKY

SEQ ID NO: 207 - protein, 20 aa, synthetic construct
  REGION 1..20: note = Description of Artificial Sequence: Cyclic peptide
YCEENYLGPEQYQYFIYFKY

SEQ ID NO: 208 - protein, 20 aa, synthetic construct
  REGION 1..20: note = Description of Artificial Sequence: Cyclic peptide
YCEENYLLPEQYQYFIYFKY

SEQ ID NO: 209 - protein, 20 aa, synthetic construct
  REGION 1..20: note = Description of Artificial Sequence: Cyclic peptide
YCEENYLIPEQYQYFIYFKY

SEQ ID NO: 210 - protein, 20 aa, synthetic construct
  REGION 1..20: note = Description of Artificial Sequence: Cyclic peptide
YCEENYLVPEQYQYFIYFKY

SEQ ID NO: 211 - protein, 20 aa, synthetic construct
  REGION 1..20: note = Description of Artificial Sequence: Cyclic peptide
YCEENYLFPEQYQYFIYFKY

SEQ ID NO: 212 - protein, 20 aa, synthetic construct
  REGION 1..20: note = Description of Artificial Sequence: Cyclic peptide
YCEENYLYPEQYQYFIYFKY

SEQ ID NO: 213 - protein, 20 aa, synthetic construct
  REGION 1..20: note = Description of Artificial Sequence: Cyclic peptide
YCEENYLWPEQYQYFIYFKY

SEQ ID NO: 214 - protein, 20 aa, synthetic construct
  REGION 1..20: note = Description of Artificial Sequence: Cyclic peptide
YCEENYLNPEQYQYFIYFKY

SEQ ID NO: 215 - protein, 20 aa, synthetic construct
  REGION 1..20: note = Description of Artificial Sequence: Cyclic peptide
YCEENYLQPEQYQYFIYFKY

SEQ ID NO: 216 - protein, 20 aa, synthetic construct
  REGION 1..20: note = Description of Artificial Sequence: Cyclic peptide
YCEENYLSPEQYQYFIYFKY

SEQ ID NO: 217 - protein, 20 aa, synthetic construct
  REGION 1..20: note = Description of Artificial Sequence: Cyclic peptide
YCEENYLTPEQYQYFIYFKY

SEQ ID NO: 218 - protein, 20 aa, synthetic construct
  REGION 1..20: note = Description of Artificial Sequence: Cyclic peptide
YCEENYLEPEQYQYFIYFKY

SEQ ID NO: 219 - protein, 20 aa, synthetic construct
  REGION 1..20: note = Description of Artificial Sequence: Cyclic peptide
YCEENYLRPEQYQYFIYFKY

SEQ ID NO: 220 - protein, 20 aa, synthetic construct
  REGION 1..20: note = Description of Artificial Sequence: Cyclic peptide
YCEENYLHPEQYQYFIYFKY

SEQ ID NO: 221 - protein, 20 aa, synthetic construct
  REGION 1..20: note = Description of Artificial Sequence: Cyclic peptide
YCEENYLDGEQYQYFIYFKY

SEQ ID NO: 222 - protein, 20 aa, synthetic construct
  REGION 1..20: note = Description of Artificial Sequence: Cyclic peptide
YCEENYLDLEQYQYFIYFKY

SEQ ID NO: 223 - protein, 20 aa, synthetic construct
  REGION 1..20: note = Description of Artificial Sequence: Cyclic peptide
YCEENYLDIEQYQYFIYFKY

SEQ ID NO: 224 - protein, 20 aa, synthetic construct
  REGION 1..20: note = Description of Artificial Sequence: Cyclic peptide
YCEENYLDVEQYQYFIYFKY

SEQ ID NO: 225 - protein, 20 aa, synthetic construct
  REGION 1..20: note = Description of Artificial Sequence: Cyclic peptide
YCEENYLDFEQYQYFIYFKY

SEQ ID NO: 226 - protein, 20 aa, synthetic construct
  REGION 1..20: note = Description of Artificial Sequence: Cyclic peptide
YCEENYLDYEQYQYFIYFKY

SEQ ID NO: 227 - protein, 20 aa, synthetic construct
  REGION 1..20: note = Description of Artificial Sequence: Cyclic peptide
YCEENYLDWEQYQYFIYFKY

SEQ ID NO: 228 - protein, 20 aa, synthetic construct
  REGION 1..20: note = Description of Artificial Sequence: Cyclic peptide
YCEENYLDNEQYQYFIYFKY

SEQ ID NO: 229 - protein, 20 aa, synthetic construct
  REGION 1..20: note = Description of Artificial Sequence: Cyclic peptide
YCEENYLDQEQYQYFIYFKY

SEQ ID NO: 230 - protein, 20 aa, synthetic construct
  REGION 1..20: note = Description of Artificial Sequence: Cyclic peptide
YCEENYLDSEQYQYFIYFKY

SEQ ID NO: 231 - protein, 20 aa, synthetic construct
  REGION 1..20: note = Description of Artificial Sequence: Cyclic peptide
YCEENYLDTEQYQYFIYFKY

SEQ ID NO: 232 - protein, 20 aa, synthetic construct
  REGION 1..20: note = Description of Artificial Sequence: Cyclic peptide
YCEENYLDDEQYQYFIYFKY

SEQ ID NO: 233 - protein, 20 aa, synthetic construct
  REGION 1..20: note = Description of Artificial Sequence: Cyclic peptide
YCEENYLDEEQYQYFIYFKY

SEQ ID NO: 234 - protein, 20 aa, synthetic construct
  REGION 1..20: note = Description of Artificial Sequence: Cyclic peptide
YCEENYLDREQYQYFIYFKY

SEQ ID NO: 235 - protein, 20 aa, synthetic construct
  REGION 1..20: note = Description of Artificial Sequence: Cyclic peptide
YCEENYLDHEQYQYFIYFKY

SEQ ID NO: 236 - protein, 20 aa, synthetic construct
  REGION 1..20: note = Description of Artificial Sequence: Cyclic peptide
YCEENYLDPGQYQYFIYFKY

SEQ ID NO: 237 - protein, 20 aa, synthetic construct
  REGION 1..20: note = Description of Artificial Sequence: Cyclic peptide
YCEENYLDPPQYQYFIYFKY

SEQ ID NO: 238 - protein, 20 aa, synthetic construct
  REGION 1..20: note = Description of Artificial Sequence: Cyclic peptide
YCEENYLDPLQYQYFIYFKY

SEQ ID NO: 239 - protein, 20 aa, synthetic construct
  REGION 1..20: note = Description of Artificial Sequence: Cyclic peptide
YCEENYLDPIQYQYFIYFKY

SEQ ID NO: 240 - protein, 20 aa, synthetic construct
  REGION 1..20: note = Description of Artificial Sequence: Cyclic peptide
YCEENYLDPVQYQYFIYFKY

SEQ ID NO: 241 - protein, 20 aa, synthetic construct
  REGION 1..20: note = Description of Artificial Sequence: Cyclic peptide
YCEENYLDPFQYQYFIYFKY

SEQ ID NO: 242 - protein, 20 aa, synthetic construct
  REGION 1..20: note = Description of Artificial Sequence: Cyclic peptide
YCEENYLDPYQYQYFIYFKY

SEQ ID NO: 243 - protein, 20 aa, synthetic construct
  REGION 1..20: note = Description of Artificial Sequence: Cyclic peptide
YCEENYLDPWQYQYFIYFKY

SEQ ID NO: 244 - protein, 20 aa, synthetic construct
  REGION 1..20: note = Description of Artificial Sequence: Cyclic peptide
YCEENYLDPNQYQYFIYFKY

SEQ ID NO: 245 - protein, 20 aa, synthetic construct
  REGION 1..20: note = Description of Artificial Sequence: Cyclic peptide
YCEENYLDPQQYQYFIYFKY

SEQ ID NO: 246 - protein, 20 aa, synthetic construct
  REGION 1..20: note = Description of Artificial Sequence: Cyclic peptide
YCEENYLDPSQYQYFIYFKY

SEQ ID NO: 247 - protein, 20 aa, synthetic construct
  REGION 1..20: note = Description of Artificial Sequence: Cyclic peptide
YCEENYLDPTQYQYFIYFKY

SEQ ID NO: 248 - protein, 20 aa, synthetic construct
  REGION 1..20: note = Description of Artificial Sequence: Cyclic peptide
YCEENYLDPDQYQYFIYFKY

SEQ ID NO: 249 - protein, 20 aa, synthetic construct
  REGION 1..20: note = Description of Artificial Sequence: Cyclic peptide
YCEENYLDPRQYQYFIYFKY

SEQ ID NO: 250 - protein, 20 aa, synthetic construct
  REGION 1..20: note = Description of Artificial Sequence: Cyclic peptide
YCEENYLDPHQYQYFIYFKY

SEQ ID NO: 251 - protein, 20 aa, synthetic construct
  REGION 1..20: note = Description of Artificial Sequence: Cyclic peptide
YCEENYLDPEHYQYFIYFKY

SEQ ID NO: 252 - protein, 20 aa, synthetic construct
  REGION 1..20: note = Description of Artificial Sequence: Cyclic peptide
YCEENYLDPEQLQYFIYFKY

SEQ ID NO: 253 - protein, 20 aa, synthetic construct
  REGION 1..20: note = Description of Artificial Sequence: Cyclic peptide
YCEENYLDPEQIQYFIYFKY

SEQ ID NO: 254 - protein, 20 aa, synthetic construct
  REGION 1..20: note = Description of Artificial Sequence: Cyclic peptide
YCEENYLDPEQFQYFIYFKY

SEQ ID NO: 255 - protein, 20 aa, synthetic construct
  REGION 1..20: note = Description of Artificial Sequence: Cyclic peptide
YCEENYLDPEQWQYFIYFKY

SEQ ID NO: 256 - protein, 20 aa, synthetic construct
  REGION 1..20: note = Description of Artificial Sequence: Cyclic peptide
YCEENYLDPEQHQYFIYFKY

SEQ ID NO: 257 - protein, 20 aa, synthetic construct
  REGION 1..20: note = Description of Artificial Sequence: Cyclic peptide
YCEENYLDPEQYGYFIYFKY

SEQ ID NO: 258 - protein, 20 aa, synthetic construct
  REGION 1..20: note = Description of Artificial Sequence: Cyclic peptide
YCEENYLDPEQYLYFIYFKY

SEQ ID NO: 259 - protein, 20 aa, synthetic construct
  REGION 1..20: note = Description of Artificial Sequence: Cyclic peptide
YCEENYLDPEQYIYFIYFKY

SEQ ID NO: 260 - protein, 20 aa, synthetic construct
  REGION 1..20: note = Description of Artificial Sequence: Cyclic peptide
YCEENYLDPEQYVYFIYFKY

SEQ ID NO: 261 - protein, 20 aa, synthetic construct
  REGION 1..20: note = Description of Artificial Sequence: Cyclic peptide
YCEENYLDPEQYFYFIYFKY

SEQ ID NO: 262 - protein, 20 aa, synthetic construct
  REGION 1..20: note = Description of Artificial Sequence: Cyclic peptide
YCEENYLDPEQYYYFIYFKY

SEQ ID NO: 263 - protein, 20 aa, synthetic construct
  REGION 1..20: note = Description of Artificial Sequence: Cyclic peptide
YCEENYLDPEQYWYFIYFKY

SEQ ID NO: 264 - protein, 20 aa, synthetic construct
  REGION 1..20: note = Description of Artificial Sequence: Cyclic peptide
YCEENYLDPEQYNYFIYFKY

SEQ ID NO: 265 - protein, 20 aa, synthetic construct
  REGION 1..20: note = Description of Artificial Sequence: Cyclic peptide
YCEENYLDPEQYSYFIYFKY

SEQ ID NO: 266 - protein, 20 aa, synthetic construct
  REGION 1..20: note = Description of Artificial Sequence: Cyclic peptide
YCEENYLDPEQYTYFIYFKY

SEQ ID NO: 267 - protein, 20 aa, synthetic construct
  REGION 1..20: note = Description of Artificial Sequence: Cyclic peptide
YCEENYLDPEQYDYFIYFKY

SEQ ID NO: 268 - protein, 20 aa, synthetic construct
  REGION 1..20: note = Description of Artificial Sequence: Cyclic peptide
YCEENYLDPEQYEYFIYFKY

SEQ ID NO: 269 - protein, 20 aa, synthetic construct
  REGION 1..20: note = Description of Artificial Sequence: Cyclic peptide
YCEENYLDPEQYRYFIYFKY

SEQ ID NO: 270 - protein, 20 aa, synthetic construct
  REGION 1..20: note = Description of Artificial Sequence: Cyclic peptide
YCEENYLDPEQYHYFIYFKY

SEQ ID NO: 271 - protein, 20 aa, synthetic construct
  REGION 1..20: note = Description of Artificial Sequence: Cyclic peptide
YCEENYLDPEQYQIFIYFKY

SEQ ID NO: 272 - protein, 20 aa, synthetic construct
  REGION 1..20: note = Description of Artificial Sequence: Cyclic peptide
YCEENYLDPEQYQFFIYFKY

SEQ ID NO: 273 - protein, 20 aa, synthetic construct
  REGION 1..20: note = Description of Artificial Sequence: Cyclic peptide
YCEENYLDPEQYQNFIYFKY

SEQ ID NO: 274 - protein, 20 aa, synthetic construct
  REGION 1..20: note = Description of Artificial Sequence: Cyclic peptide
YCEENYLDPEQYQHFIYFKY

SEQ ID NO: 275 - protein, 20 aa, synthetic construct
  REGION 1..20: note = Description of Artificial Sequence: Cyclic peptide
YCEENYLDPEQYQYLIYFKY

SEQ ID NO: 276 - protein, 20 aa, synthetic construct
  REGION 1..20: note = Description of Artificial Sequence: Cyclic peptide
YCEENYLDPEQYQYYIYFKY

SEQ ID NO: 277 - protein, 20 aa, synthetic construct
  REGION 1..20: note = Description of Artificial Sequence: Cyclic peptide
YCEENYLDPEQYQYFGYFKY

SEQ ID NO: 278 - protein, 20 aa, synthetic construct
  REGION 1..20: note = Description of Artificial Sequence: Cyclic peptide
YCEENYLDPEQYQYFLYFKY

SEQ ID NO: 279 - protein, 20 aa, synthetic construct
  REGION 1..20: note = Description of Artificial Sequence: Cyclic peptide
YCEENYLDPEQYQYFVYFKY

SEQ ID NO: 280 - protein, 20 aa, synthetic construct
  REGION 1..20: note = Description of Artificial Sequence: Cyclic peptide
YCEENYLDPEQYQYFFYFKY

SEQ ID NO: 281 - protein, 20 aa, synthetic construct
  REGION 1..20: note = Description of Artificial Sequence: Cyclic peptide
YCEENYLDPEQYQYFYYFKY

SEQ ID NO: 282 - protein, 20 aa, synthetic construct
  REGION 1..20: note = Description of Artificial Sequence: Cyclic peptide
YCEENYLDPEQYQYFWYFKY

SEQ ID NO: 283 - protein, 20 aa, synthetic construct
  REGION 1..20: note = Description of Artificial Sequence: Cyclic peptide
YCEENYLDPEQYQYFNYFKY

SEQ ID NO: 284 - protein, 20 aa, synthetic construct
  REGION 1..20: note = Description of Artificial Sequence: Cyclic peptide
YCEENYLDPEQYQYFQYFKY

SEQ ID NO: 285 - protein, 20 aa, synthetic construct
  REGION 1..20: note = Description of Artificial Sequence: Cyclic peptide
YCEENYLDPEQYQYFSYFKY

SEQ ID NO: 286 - protein, 20 aa, synthetic construct
  REGION 1..20: note = Description of Artificial Sequence: Cyclic peptide
YCEENYLDPEQYQYFTYFKY

SEQ ID NO: 287 - protein, 20 aa, synthetic construct
  REGION 1..20: note = Description of Artificial Sequence: Cyclic peptide
YCEENYLDPEQYQYFDYFKY

SEQ ID NO: 288 - protein, 20 aa, synthetic construct
  REGION 1..20: note = Description of Artificial Sequence: Cyclic peptide
YCEENYLDPEQYQYFEYFKY

SEQ ID NO: 289 - protein, 20 aa, synthetic construct
  REGION 1..20: note = Description of Artificial Sequence: Cyclic peptide
YCEENYLDPEQYQYFRYFKY

SEQ ID NO: 290 - protein, 20 aa, synthetic construct
  REGION 1..20: note = Description of Artificial Sequence: Cyclic peptide
YCEENYLDPEQYQYFHYFKY

SEQ ID NO: 291 - protein, 20 aa, synthetic construct
  REGION 1..20: note = Description of Artificial Sequence: Cyclic peptide
YCEENYLDPEQYQYFIGFKY

SEQ ID NO: 292 - protein, 20 aa, synthetic construct
  REGION 1..20: note = Description of Artificial Sequence: Cyclic peptide
YCEENYLDPEQYQYFIPFKY

SEQ ID NO: 293 - protein, 20 aa, synthetic construct
  REGION 1..20: note = Description of Artificial Sequence: Cyclic peptide
YCEENYLDPEQYQYFILFKY

SEQ ID NO: 294 - protein, 20 aa, synthetic construct
  REGION 1..20: note = Description of Artificial Sequence: Cyclic peptide
YCEENYLDPEQYQYFIIFKY

SEQ ID NO: 295 - protein, 20 aa, synthetic construct
  REGION 1..20: note = Description of Artificial Sequence: Cyclic peptide
YCEENYLDPEQYQYFIVFKY

SEQ ID NO: 296 - protein, 20 aa, synthetic construct
  REGION 1..20: note = Description of Artificial Sequence: Cyclic peptide
YCEENYLDPEQYQYFIFFKY

SEQ ID NO: 297 - protein, 20 aa, synthetic construct
  REGION 1..20: note = Description of Artificial Sequence: Cyclic peptide
YCEENYLDPEQYQYFIWFKY

SEQ ID NO: 298 - protein, 20 aa, synthetic construct
  REGION 1..20: note = Description of Artificial Sequence: Cyclic peptide
YCEENYLDPEQYQYFINFKY

SEQ ID NO: 299 - protein, 20 aa, synthetic construct
  REGION 1..20: note = Description of Artificial Sequence: Cyclic peptide
YCEENYLDPEQYQYFIQFKY

SEQ ID NO: 300 - protein, 20 aa, synthetic construct
  REGION 1..20: note = Description of Artificial Sequence: Cyclic peptide
YCEENYLDPEQYQYFISFKY

SEQ ID NO: 301 - protein, 20 aa, synthetic construct
  REGION 1..20: note = Description of Artificial Sequence: Cyclic peptide
YCEENYLDPEQYQYFITFKY

SEQ ID NO: 302 - protein, 20 aa, synthetic construct
  REGION 1..20: note = Description of Artificial Sequence: Cyclic peptide
YCEENYLDPEQYQYFIDFKY

SEQ ID NO: 303 - protein, 20 aa, synthetic construct
  REGION 1..20: note = Description of Artificial Sequence: Cyclic peptide
YCEENYLDPEQYQYFIEFKY

SEQ ID NO: 304 - protein, 20 aa, synthetic construct
  REGION 1..20: note = Description of Artificial Sequence: Cyclic peptide
YCEENYLDPEQYQYFIRFKY

SEQ ID NO: 305 - protein, 20 aa, synthetic construct
  REGION 1..20: note = Description of Artificial Sequence: Cyclic peptide
YCEENYLDPEQYQYFIHFKY

SEQ ID NO: 306 - protein, 20 aa, synthetic construct
  REGION 1..20: note = Description of Artificial Sequence: Cyclic peptide
YCEENYLDPEQYQYFIYYKY

SEQ ID NO: 307 - protein, 20 aa, synthetic construct
  REGION 1..20: note = Description of Artificial Sequence: Cyclic peptide
YCEENYLDPEQYQYFIYWKY

SEQ ID NO: 308 - protein, 20 aa, synthetic construct
  REGION 1..20: note = Description of Artificial Sequence: Cyclic peptide
YCEENYLDPEQYQYFIYFKG

SEQ ID NO: 309 - protein, 20 aa, synthetic construct
  REGION 1..20: note = Description of Artificial Sequence: Cyclic peptide
YCEENYLDPEQYQYFIYFKL

SEQ ID NO: 310 - protein, 20 aa, synthetic construct
  REGION 1..20: note = Description of Artificial Sequence: Cyclic peptide
YCEENYLDPEQYQYFIYFKI

SEQ ID NO: 311 - protein, 20 aa, synthetic construct
  REGION 1..20: note = Description of Artificial Sequence: Cyclic peptide
YCEENYLDPEQYQYFIYFKV

SEQ ID NO: 312 - protein, 20 aa, synthetic construct
  REGION 1..20: note = Description of Artificial Sequence: Cyclic peptide
YCEENYLDPEQYQYFIYFKF

SEQ ID NO: 313 - protein, 20 aa, synthetic construct
  REGION 1..20: note = Description of Artificial Sequence: Cyclic peptide
YCEENYLDPEQYQYFIYFKW

SEQ ID NO: 314 - protein, 20 aa, synthetic construct
  REGION 1..20: note = Description of Artificial Sequence: Cyclic peptide
YCEENYLDPEQYQYFIYFKN

SEQ ID NO: 315 - protein, 20 aa, synthetic construct
  REGION 1..20: note = Description of Artificial Sequence: Cyclic peptide
YCEENYLDPEQYQYFIYFKQ

SEQ ID NO: 316 - protein, 20 aa, synthetic construct
  REGION 1..20: note = Description of Artificial Sequence: Cyclic peptide
YCEENYLDPEQYQYFIYFKS

SEQ ID NO: 317 - protein, 20 aa, synthetic construct
  REGION 1..20: note = Description of Artificial Sequence: Cyclic peptide
YCEENYLDPEQYQYFIYFKT

SEQ ID NO: 318 - protein, 20 aa, synthetic construct
  REGION 1..20: note = Description of Artificial Sequence: Cyclic peptide
YCEENYLDPEQYQYFIYFKD

SEQ ID NO: 319 - protein, 20 aa, synthetic construct
  REGION 1..20: note = Description of Artificial Sequence: Cyclic peptide
YCEENYLDPEQYQYFIYFKE

SEQ ID NO: 320 - protein, 20 aa, synthetic construct
  REGION 1..20: note = Description of Artificial Sequence: Cyclic peptide
YCEENYLDPEQYQYFIYFKR

SEQ ID NO: 321 - protein, 20 aa, synthetic construct
  REGION 1..20: note = Description of Artificial Sequence: Cyclic peptide
YCEENYLDPEQYQYFIYFKH

SEQ ID NO: 322 - protein, 20 aa, synthetic construct
  REGION 1..20: note = Description of Artificial Sequence: Cyclic peptide
ACEENYLDPEQYQYFIYFKY

SEQ ID NO: 323 - protein, 20 aa, synthetic construct
  REGION 1..20: note = Description of Artificial Sequence: Cyclic peptide
YCAENYLDPEQYQYFIYFKY

SEQ ID NO: 324 - protein, 20 aa, synthetic construct
  REGION 1..20: note = Description of Artificial Sequence: Cyclic peptide
YCEANYLDPEQYQYFIYFKY

SEQ ID NO: 325 - protein, 20 aa, synthetic construct
  REGION 1..20: note = Description of Artificial Sequence: Cyclic peptide
YCEEAYLDPEQYQYFIYFKY

SEQ ID NO: 326 - protein, 20 aa, synthetic construct
  REGION 1..20: note = Description of Artificial Sequence: Cyclic peptide
YCEENALDPEQYQYFIYFKY

SEQ ID NO: 327 - protein, 20 aa, synthetic construct
  REGION 1..20: note = Description of Artificial Sequence: Cyclic peptide
YCEENYADPEQYQYFIYFKY

SEQ ID NO: 328 - protein, 20 aa, synthetic construct
  REGION 1..20: note = Description of Artificial Sequence: Cyclic peptide
YCEENYLAPEQYQYFIYFKY

SEQ ID NO: 329 - protein, 20 aa, synthetic construct
  REGION 1..20: note = Description of Artificial Sequence: Cyclic peptide
YCEENYLDAEQYQYFIYFKY

SEQ ID NO: 330 - protein, 20 aa, synthetic construct
  REGION 1..20: note = Description of Artificial Sequence: Cyclic peptide
YCEENYLDPAQYQYFIYFKY

SEQ ID NO: 331 - protein, 20 aa, synthetic construct
  REGION 1..20: note = Description of Artificial Sequence: Cyclic peptide
YCEENYLDPEQYAYFIYFKY

SEQ ID NO: 332 - protein, 20 aa, synthetic construct
  REGION 1..20: note = Description of Artificial Sequence: Cyclic peptide
YCEENYLDPEQYQYFAYFKY

SEQ ID NO: 333 - protein, 20 aa, synthetic construct
  REGION 1..20: note = Description of Artificial Sequence: Cyclic peptide
YCEENYLDPEQYQYFIAFKY

SEQ ID NO: 334 - protein, 20 aa, synthetic construct
  REGION 1..20: note = Description of Artificial Sequence: Cyclic peptide
YCEENYLDPEQYQYFIYFKA

SEQ ID NO: 335 - protein, 20 aa, synthetic construct
  REGION 1..20: note = Description of Artificial Sequence: Cyclic peptide
KCEENYLDPEQYQYFIYFKY

SEQ ID NO: 336 - protein, 20 aa, synthetic construct
  REGION 1..20: note = Description of Artificial Sequence: Cyclic peptide
YCKENYLDPEQYQYFIYFKY

SEQ ID NO: 337 - protein, 20 aa, synthetic construct
  REGION 1..20: note = Description of Artificial Sequence: Cyclic peptide
YCEKNYLDPEQYQYFIYFKY

SEQ ID NO: 338 - protein, 20 aa, synthetic construct
  REGION 1..20: note = Description of Artificial Sequence: Cyclic peptide
YCEENKLDPEQYQYFIYFKY

SEQ ID NO: 339 - protein, 20 aa, synthetic construct
  REGION 1..20: note = Description of Artificial Sequence: Cyclic peptide
YCEENYKDPEQYQYFIYFKY

SEQ ID NO: 340 - protein, 20 aa, synthetic construct
  REGION 1..20: note = Description of Artificial Sequence: Cyclic peptide
YCEENYLKPEQYQYFIYFKY

SEQ ID NO: 341 - protein, 20 aa, synthetic construct
  REGION 1..20: note = Description of Artificial Sequence: Cyclic peptide
YCEENYLDKEQYQYFIYFKY

SEQ ID NO: 342 - protein, 20 aa, synthetic construct
  REGION 1..20: note = Description of Artificial Sequence: Cyclic peptide
YCEENYLDPKQYQYFIYFKY

SEQ ID NO: 343 - protein, 20 aa, synthetic construct
  REGION 1..20: note = Description of Artificial Sequence: Cyclic peptide
YCEENYLDPEQYKYFIYFKY

SEQ ID NO: 344 - protein, 20 aa, synthetic construct
  REGION 1..20: note = Description of Artificial Sequence: Cyclic peptide
YCEENYLDPEQYQYFKYFKY

SEQ ID NO: 345 - protein, 20 aa, synthetic construct
  REGION 1..20: note = Description of Artificial Sequence: Cyclic peptide
YCEENYLDPEQYQYFIKFKY

SEQ ID NO: 346 - protein, 20 aa, synthetic construct
  REGION 1..20: note = Description of Artificial Sequence: Cyclic peptide
YCEENYLDPEQYQYFIYFKK

SEQ ID NO: 347 - protein, 20 aa, synthetic construct
  REGION 1..20: note = Description of Artificial Sequence: Cyclic peptide
MCEENYLDPEQYQYFIYFKY

SEQ ID NO: 348 - protein, 20 aa, synthetic construct
  REGION 1..20: note = Description of Artificial Sequence: Cyclic peptide
YCMENYLDPEQYQYFIYFKY

SEQ ID NO: 349 - protein, 20 aa, synthetic construct
  REGION 1..20: note = Description of Artificial Sequence: Cyclic peptide
YCEMNYLDPEQYQYFIYFKY

SEQ ID NO: 350 - protein, 20 aa, synthetic construct
  REGION 1..20: note = Description of Artificial Sequence: Cyclic peptide
YCEENMLDPEQYQYFIYFKY

SEQ ID NO: 351 - protein, 20 aa, synthetic construct
  REGION 1..20: note = Description of Artificial Sequence: Cyclic peptide
YCEENYMDPEQYQYFIYFKY

SEQ ID NO: 352 - protein, 20 aa, synthetic construct
  REGION 1..20: note = Description of Artificial Sequence: Cyclic peptide
YCEENYLMPEQYQYFIYFKY

SEQ ID NO: 353 - protein, 20 aa, synthetic construct
  REGION 1..20: note = Description of Artificial Sequence: Cyclic peptide
YCEENYLDMEQYQYFIYFKY

SEQ ID NO: 354 - protein, 20 aa, synthetic construct
  REGION 1..20: note = Description of Artificial Sequence: Cyclic peptide
YCEENYLDPMQYQYFIYFKY

SEQ ID NO: 355 - protein, 20 aa, synthetic construct
  REGION 1..20: note = Description of Artificial Sequence: Cyclic peptide
YCEENYLDPEQMQYFIYFKY

SEQ ID NO: 356 - protein, 20 aa, synthetic construct
  REGION 1..20: note = Description of Artificial Sequence: Cyclic peptide
YCEENYLDPEQYMYFIYFKY

SEQ ID NO: 357 - protein, 20 aa, synthetic construct
  REGION 1..20: note = Description of Artificial Sequence: Cyclic peptide
YCEENYLDPEQYQMFIYFKY

SEQ ID NO: 358 - protein, 20 aa, synthetic construct
  REGION 1..20: note = Description of Artificial Sequence: Cyclic peptide
YCEENYLDPEQYQYFMYFKY

SEQ ID NO: 359 - protein, 20 aa, synthetic construct
  REGION 1..20: note = Description of Artificial Sequence: Cyclic peptide
YCEENYLDPEQYQYFIMFKY

SEQ ID NO: 360 - protein, 20 aa, synthetic construct
  REGION 1..20: note = Description of Artificial Sequence: Cyclic peptide
YCEENYLDPEQYQYFIYFKM

SEQ ID NO: 361 - protein, 12 aa, synthetic construct
  REGION 1..12: note = Description of Artificial Sequence: Cyclic peptide
QCYYLYWYLYKI

SEQ ID NO: 362 - protein, 13 aa, synthetic construct
  REGION 1..13: note = Description of Artificial Sequence: Cyclic peptide
LCYLYQYLYTTKY

SEQ ID NO: 363 - protein, 13 aa, synthetic construct
  REGION 1..13: note = Description of Artificial Sequence: Cyclic peptide
LCYLYQYIYTAKF

SEQ ID NO: 364 - protein, 13 aa, synthetic construct
  REGION 1..13: note = Description of Artificial Sequence: Cyclic peptide
QCLQYLYQYLFKI

SEQ ID NO: 365 - protein, 13 aa, synthetic construct
  REGION 1..13: note = Description of Artificial Sequence: Cyclic peptide
LCYLYQYLYQAKF

SEQ ID NO: 366 - protein, 14 aa, synthetic construct
  REGION 1..14: note = Description of Artificial Sequence: Cyclic peptide
DCQQYYLYLYLWKI

SEQ ID NO: 367 - protein, 14 aa, synthetic construct
  REGION 1..14: note = Description of Artificial Sequence: Cyclic peptide
HCQLEYLYTYVLKI

SEQ ID NO: 368 - protein, 14 aa, synthetic construct
  REGION 1..14: note = Description of Artificial Sequence: Cyclic peptide
QCLIQDLYAYIFKL

SEQ ID NO: 369 - protein, 14 aa, synthetic construct
  REGION 1..14: note = Description of Artificial Sequence: Cyclic peptide
DCLQFLYLYLYQKT

SEQ ID NO: 370 - protein, 15 aa, synthetic construct
  REGION 1..15: note = Description of Artificial Sequence: Cyclic peptide
DCQLYYLYQYVLTKV

SEQ ID NO: 371 - protein, 15 aa, synthetic construct
  REGION 1..15: note = Description of Artificial Sequence: Cyclic peptide
DCQLWYLYQYLIVKA

SEQ ID NO: 372 - protein, 15 aa, synthetic construct
  REGION 1..15: note = Description of Artificial Sequence: Cyclic peptide
QCEQLKYLYQYVLKL

SEQ ID NO: 373 - protein, 15 aa, synthetic construct
  REGION 1..15: note = Description of Artificial Sequence: Cyclic peptide
QCYNYQYIYQYIYKI

SEQ ID NO: 374 - protein, 15 aa, synthetic construct
  REGION 1..15: note = Description of Artificial Sequence: Cyclic peptide
QCLQDLYRYLYLLKA

SEQ ID NO: 375 - protein, 15 aa, synthetic construct
  REGION 1..15: note = Description of Artificial Sequence: Cyclic peptide
DCLQFIYQYLYTVKI

SEQ ID NO: 376 - protein, 15 aa, synthetic construct
  REGION 1..15: note = Description of Artificial Sequence: Cyclic peptide
QCIQDLYLYLYFLKT

SEQ ID NO: 377 - protein, 15 aa, synthetic construct
  REGION 1..15: note = Description of Artificial Sequence: Cyclic peptide
HCLHYLYQYLYTVKY

SEQ ID NO: 378 - protein, 16 aa, synthetic construct
  REGION 1..16: note = Description of Artificial Sequence: Cyclic peptide
QCPRQLYYLYLYLSKI

SEQ ID NO: 379 - protein, 16 aa, synthetic construct
  REGION 1..16: note = Description of Artificial Sequence: Cyclic peptide
NCQLYYTYLYLHTLKF

SEQ ID NO: 380 - protein, 16 aa, synthetic construct
  REGION 1..16: note = Description of Artificial Sequence: Cyclic peptide
YCPPQLVYLYQYLYKL

SEQ ID NO: 381 - protein, 16 aa, synthetic construct
  REGION 1..16: note = Description of Artificial Sequence: Cyclic peptide
VCQEYYLYQYVYELKY

SEQ ID NO: 382 - protein, 16 aa, synthetic construct
  REGION 1..16: note = Description of Artificial Sequence: Cyclic peptide
PCDRQLYYLYQYIHKT

SEQ ID NO: 383 - protein, 16 aa, synthetic construct
  REGION 1..16: note = Description of Artificial Sequence: Cyclic peptide
QCQLYYLYQYAYALKV

SEQ ID NO: 384 - protein, 16 aa, synthetic construct
  REGION 1..16: note = Description of Artificial Sequence: Cyclic peptide
QCQLYYLYQYTIAIKT

SEQ ID NO: 385 - protein, 16 aa, synthetic construct
  REGION 1..16: note = Description of Artificial Sequence: Cyclic peptide
QCAYYHLYQYLHQLKV

SEQ ID NO: 386 - protein, 20 aa, synthetic construct
  REGION 1..20: note = Description of Artificial Sequence: Cyclic peptide
RCHHNFHHARQWGFFHHYKR

SEQ ID NO: 387 - protein, 20 aa, synthetic construct
  REGION 1..20: note = Description of Artificial Sequence: Cyclic peptide
RCHHNFHHARQHRFFHHYKR

SEQ ID NO: 388 - protein, 20 aa, synthetic construct
  REGION 1..20: note = Description of Artificial Sequence: Cyclic peptide
RCHHNFHHARQHGFFYHYKR

SEQ ID NO: 389 - protein, 20 aa, synthetic construct
  REGION 1..20: note = Description of Artificial Sequence: Cyclic peptide
RCHHNFHHARQHGFFWHYKR

SEQ ID NO: 390 - protein, 20 aa, synthetic construct
  REGION 1..20: note = Description of Artificial Sequence: Cyclic peptide
YCEENYLDPEQYQYFHYFKR

SEQ ID NO: 391 - protein, 20 aa, synthetic construct
  REGION 1..20: note = Description of Artificial Sequence: Cyclic peptide
YCEENYLDPEQYQYFHYFKH

SEQ ID NO: 392 - protein, 20 aa, synthetic construct
  REGION 1..20: note = Description of Artificial Sequence: Cyclic peptide
YCHENYLDPEQYQYFHYFKY

SEQ ID NO: 393 - protein, 20 aa, synthetic construct
  REGION 1..20: note = Description of Artificial Sequence: Cyclic peptide
YCHENYLDPEQHQYFHYFKY

SEQ ID NO: 394 - protein, 20 aa, synthetic construct
  REGION 1..20: note = Description of Artificial Sequence: Cyclic peptide
YCHENYLDPEQYQYFHYFKR

SEQ ID NO: 395 - protein, 20 aa, synthetic construct
  REGION 1..20: note = Description of Artificial Sequence: Cyclic peptide
YCHENYLDPEQYQYFHYFKH

SEQ ID NO: 396 - protein, 20 aa, synthetic construct
  REGION 1..20: note = Description of Artificial Sequence: Cyclic peptide
YCEENYLDPEQHQYFIYFKR

SEQ ID NO: 397 - protein, 20 aa, synthetic construct
  REGION 1..20: note = Description of Artificial Sequence: Cyclic peptide
YCEENYLDPEQHQYFIYFKH

SEQ ID NO: 398 - protein, 20 aa, synthetic construct
  REGION 1..20: note = Description of Artificial Sequence: Cyclic peptide
YCHENYLDPEQHQYFIYFKR

SEQ ID NO: 399 - protein, 20 aa, synthetic construct
  REGION 1..20: note = Description of Artificial Sequence: Cyclic peptide
QKPQNFINPVQWRYFQHYCN

SEQ ID NO: 400 - protein, 21 aa, synthetic construct
  REGION 1..21: note = Description of Artificial Sequence: Cyclic peptide
VCQQDNYFYPQQWFFFVHYKH

SEQ ID NO: 401 - protein, 21 aa, synthetic construct
  REGION 1..21: note = Description of Artificial Sequence: Cyclic peptide
QCQFLNYVNHVQWHYFWVFKS

SEQ ID NO: 402 - protein, 21 aa, synthetic construct
  REGION 1..21: note = Description of Artificial Sequence: Cyclic peptide
PCEVYNYWYPTQWFFFTQFKK

SEQ ID NO: 403 - protein, 21 aa, synthetic construct
  REGION 1..21: note = Description of Artificial Sequence: Cyclic peptide
ACRRANWIHPIQWFFFHVYKH

SEQ ID NO: 404 - protein, 21 aa, synthetic construct
  REGION 1..21: note = Description of Artificial Sequence: Cyclic peptide
DCIRPYDQLQLIYQYLYQLKK

SEQ ID NO: 405 - protein, 21 aa, synthetic construct
  REGION 1..21: note = Description of Artificial Sequence: Cyclic peptide
QCLTQRVYLRQLAYYRLYRKI

SEQ ID NO: 406 - protein, 21 aa, synthetic construct
  REGION 1..21: note = Description of Artificial Sequence: Cyclic peptide
PCEQQNFHSVIQWHFFAQYKN

SEQ ID NO: 407 - protein, 21 aa, synthetic construct
  REGION 1..21: note = Description of Artificial Sequence: Cyclic peptide
LCVQGNYQNPTQWYYFQLYKW

SEQ ID NO: 408 - protein, 21 aa, synthetic construct
  REGION 1..21: note = Description of Artificial Sequence: Cyclic peptide
HCSQHQTTYYQIYAYLHAIKI

SEQ ID NO: 409 - protein, 22 aa, synthetic construct
  REGION 1..22: note = Description of Artificial Sequence: Cyclic peptide
LCNNWENYFDWLQWSYYIAYKE

SEQ ID NO: 410 - protein, 22 aa, synthetic construct
  REGION 1..22: note = Description of Artificial Sequence: Cyclic peptide
WCQESSNYLAPLQWYFFNWYKT

SEQ ID NO: 411 - protein, 22 aa, synthetic construct
  REGION 1..22: note = Description of Artificial Sequence: Cyclic peptide
TCVDKDNWYNHVQWQYFFLYKQ

SEQ ID NO: 412 - protein, 22 aa, synthetic construct
  REGION 1..22: note = Description of Artificial Sequence: Cyclic peptide
QCEYALQYYRFYVAQRHWVDKL

SEQ ID NO: 413 - protein, 22 aa, synthetic construct
  REGION 1..22: note = Description of Artificial Sequence: Cyclic peptide
QCDQDAIQWVYDLQYYRVWHKV

SEQ ID NO: 414 - protein, 22 aa, synthetic construct
  REGION 1..22: note = Description of Artificial Sequence: Cyclic peptide
YCNYEWDGARRQIAYYRIFLKL

SEQ ID NO: 415 - protein, 22 aa, synthetic construct
  REGION 1..22: note = Description of Artificial Sequence: Cyclic peptide
YCDWVEVANARQLAYYTLYRKK

SEQ ID NO: 416 - protein, 22 aa, synthetic construct
  REGION 1..22: note = Description of Artificial Sequence: Cyclic peptide
LCTQFPASQRYYFALYRLWHKS

SEQ ID NO: 417 - protein, 22 aa, synthetic construct
  REGION 1..22: note = Description of Artificial Sequence: Cyclic peptide
LCQIYLYLTALQQGFEDFYPKN

SEQ ID NO: 418 - protein, 22 aa, synthetic construct
  REGION 1..22: note = Description of Artificial Sequence: Cyclic peptide
DCLRQQVYQYLYILFQNDIAKD

SEQ ID NO: 419 - protein, 22 aa, synthetic construct
  REGION 1..22: note = Description of Artificial Sequence: Cyclic peptide
DCHTREDWQIHHLYQLLYQLKY

SEQ ID NO: 420 - protein, 21 aa, synthetic construct
  REGION 1..21: note = Description of Artificial Sequence: Cyclic peptide
YCEAQPYYFQLYRLWHRQEKP

SEQ ID NO: 421 - protein, 21 aa, synthetic construct
  REGION 1..21: note = Description of Artificial Sequence: Cyclic peptide
VCLDEQQALFHQYYRITRRKV

SEQ ID NO: 422 - protein, 22 aa, synthetic construct
  REGION 1..22: note = Description of Artificial Sequence: Cyclic peptide
YCTQEQAFRQLAYYQIFRRSKS

SEQ ID NO: 423 - protein, 21 aa, synthetic construct
  REGION 1..21: note = Description of Artificial Sequence: Cyclic peptide
WCFTEGIQSTVQLTYSYLYKL

SEQ ID NO: 424 - protein, 22 aa, synthetic construct
  REGION 1..22: note = Description of Artificial Sequence: Cyclic peptide
VCTQPQQDFELIYQYLYQLAKQ

SEQ ID NO: 425 - protein, 21 aa, synthetic construct
  REGION 1..21: note = Description of Artificial Sequence: Cyclic peptide
GCGYTQLHYQHLFAWLHARKV

SEQ ID NO: 426 - protein, 21 aa, synthetic construct
  REGION 1..21: note = Description of Artificial Sequence: Cyclic peptide
PCDPLNLQQWYTAVYQLWHKR

SEQ ID NO: 427 - protein, 22 aa, synthetic construct
  REGION 1..22: note = Description of Artificial Sequence: Cyclic peptide
ECDTADYPQEWIQDVYQYLYKR

SEQ ID NO: 428 - protein, 22 aa, synthetic construct
  REGION 1..22: note = Description of Artificial Sequence: Cyclic peptide
ECDQAQQVYALIYRYLYQLQKV

SEQ ID NO: 429 - protein, 19 aa, synthetic construct
  REGION 1..19: note = Description of Artificial Sequence: Cyclic peptide
YCHENYLDPEQYQYFHYFK

SEQ ID NO: 430 - protein, 19 aa, synthetic construct
  REGION 1..19: note = Description of Artificial Sequence: Cyclic peptide
CHENYLDPEQYQYFHYFKY

SEQ ID NO: 431 - protein, 18 aa, synthetic construct
  REGION 1..18: note = Description of Artificial Sequence: Cyclic peptide
CHENYLDPEQYQYFHYFK

SEQ ID NO: 432 - protein, 18 aa, synthetic construct
  REGION 1..18: note = Description of Artificial Sequence: Cyclic peptide
CENYLDPEQYQYFHYFKY

SEQ ID NO: 433 - protein, 23 aa, synthetic construct
  REGION 1..23: note = Description of Artificial Sequence: Cyclic peptide
QXPQNFINPVQWRYFQHYKNKKK

SEQ ID NO: 434 - protein, 23 aa, synthetic construct
  REGION 1..23: note = Description of Artificial Sequence: Cyclic peptide
QXPQNFINPVQWRYFQHYXNKKK

SEQ ID NO: 435 - protein, 23 aa, synthetic construct
  REGION 1..23: note = Description of Artificial Sequence: Cyclic peptide
QXPQNFINPVQWRYFQHYXNKKK

SEQ ID NO: 436 - skipped

SEQ ID NO: 437 - protein, 23 aa, synthetic construct
  REGION 1..23: note = Description of Artificial Sequence: Cyclic peptide
QKPQNFINPVQWRYFQHYXNKKK

SEQ ID NO: 438 - protein, 23 aa, synthetic construct
  REGION 1..23: note = Description of Artificial Sequence: Cyclic peptide
QKPQNFINPVQWRYFQHYXNKKK

SEQ ID NO: 439 - protein, 23 aa, synthetic construct
  REGION 1..23: note = Description of Artificial Sequence: Cyclic peptide
QXPQNFINPVQWRYFQHYXNKKK

SEQ ID NO: 440 - protein, 23 aa, synthetic construct
  REGION 1..23: note = Description of Artificial Sequence: Cyclic peptide
QXPQNFINPVQWRYFQHYXNKKK

SEQ ID NO: 441 - protein, 23 aa, synthetic construct
  REGION 1..23: note = Description of Artificial Sequence: Cyclic peptide
QXPQNFINPVQWRYFQHYXNKKK

SEQ ID NO: 442 - protein, 23 aa, synthetic construct
  REGION 1..23: note = Description of Artificial Sequence: Cyclic peptide
YXEENYLDPEQYQYFIYFKYKKK

SEQ ID NO: 443 - protein, 23 aa, synthetic construct
  REGION 1..23: note = Description of Artificial Sequence: Cyclic peptide
YXEENYLDPEQYQYFIYFXYKKK

SEQ ID NO: 444 - protein, 23 aa, synthetic construct
  REGION 1..23: note = Description of Artificial Sequence: Cyclic peptide
YXEENYLDPEQYQYFIYFXYKKK

SEQ ID NO: 445 - skipped

SEQ ID NO: 446 - protein, 23 aa, synthetic construct
  REGION 1..23: note = Description of Artificial Sequence: Cyclic peptide
YKEENYLDPEQYQYFIYFXYKKK

SEQ ID NO: 447 - protein, 23 aa, synthetic construct
  REGION 1..23: note = Description of Artificial Sequence: Cyclic peptide
YXEENYLDPEQYQYFIYFXYKKK

SEQ ID NO: 448 - protein, 23 aa, synthetic construct
  REGION 1..23: note = Description of Artificial Sequence: Cyclic peptide
YXEENYLDPEQYQYFIYFXYKKK

SEQ ID NO: 449 - protein, 23 aa, synthetic construct
  REGION 1..23: note = Description of Artificial Sequence: Cyclic peptide
YXEENYLDPEQYQYFIYFXYKKK

SEQ ID NO: 450 - protein, 23 aa, synthetic construct
  REGION 1..23: note = Description of Artificial Sequence: Cyclic peptide
YCEENYLDPEQYQYFIYFKYKKK

SEQ ID NO: 451 - protein, 23 aa, synthetic construct
  REGION 1..23: note = Description of Artificial Sequence: Cyclic peptide
YCEENYLDPEQYQYFIYFCYKKK

SEQ ID NO: 452 - protein, 23 aa, synthetic construct
  REGION 1..23: note = Description of Artificial Sequence: Cyclic peptide
YXHENYLDPEQYQYFHYFKYKKK

SEQ ID NO: 453 - protein, 22 aa, synthetic construct
  REGION 1..22: note = Description of Artificial Sequence: Cyclic peptide
YXHENYLDPEQYQYFHYFKKKK

SEQ ID NO: 454 - protein, 22 aa, synthetic construct
  REGION 1..22: note = Description of Artificial Sequence: Cyclic peptide
XHENYLDPEQYQYFHYFKYKKK

SEQ ID NO: 455 - protein, 54 aa, synthetic construct
  REGION 1..54: note = Description of Artificial Sequence: Cyclic peptide
KCPQNFINPVQWRYFQHYKNGSGSGSSGSSSGSSKCPQNFINPVQWRYFQHYKN

SEQ ID NO: 456 - protein, 42 aa, synthetic construct
  REGION 1..42: note = Description of Artificial Sequence: Cyclic peptide
QCPQNFINPVQWRYFQHYKNKQCPQNFINPVQWRYFQHYKNK

SEQ ID NO: 457 - protein, 42 aa, synthetic construct; identical to SEQ ID NO: 456
  REGION 1..42: note = Description of Artificial Sequence: Cyclic peptide

SEQ ID NO: 458 - protein, 42 aa, synthetic construct; identical to SEQ ID NO: 456
  REGION 1..42: note = Description of Artificial Sequence: Cyclic peptide

SEQ ID NO: 459 - protein, 41 aa, synthetic construct
  REGION 1..41: note = Description of Artificial Sequence: Cyclic peptide
QCPQNFINPVQWRYFQHYKNQCPQNFINPVQWRYFQHYKNK

SEQ ID NO: 460 - protein, 42 aa, synthetic construct
  REGION 1..42: note = Description of Artificial Sequence: Cyclic peptide
YCEENYLDPEQYQYFIYFKYKYCEENYLDPEQYQYFIYFKYK

SEQ ID NO: 461 - protein, 42 aa, synthetic construct
  REGION 1..42: note = Description of Artificial Sequence: Cyclic peptide
YXHENYLDPEQYQYFHYFKYKYXHENYLDPEQYQYFHYFKYK

SEQ ID NO: 462 - protein, 42 aa, synthetic construct; identical to SEQ ID NO: 461
  REGION 1..42: note = Description of Artificial Sequence: Cyclic peptide

SEQ ID NO: 463 - protein, 42 aa, synthetic construct; identical to SEQ ID NO: 461
  REGION 1..42: note = Description of Artificial Sequence: Cyclic peptide